European Patent Specification EP 3 653 218 B1, published December 18, 2024. Title: METHODS OF TREATING OR PREVENTING RHEUMATIC DISEASE. Applicant: Mesoblast, Inc. The sequence listing filed with the application follows.

SEQUENCE LISTING (36 sequences)

SEQ ID NO: 1 - DNA, 20 bp, artificial
  oligonucleotide for amplifying GAPDH
cactgacacgttggcagtgg

SEQ ID NO: 2 - DNA, 20 bp, artificial
  oligonucleotide for amplifying GAPDH
catggagaaggctggggctc

SEQ ID NO: 3 - DNA, 20 bp, artificial
  oligonucleotide for amplifying SDF-1
gagacccgcgctcgtccgcc

SEQ ID NO: 4 - DNA, 21 bp, artificial
  oligonucleotide for amplifying SDF-1
gctggactcctactgtaaggg

SEQ ID NO: 5 - DNA, 22 bp, artificial
  oligonucleotide for amplifying IL-1beta
aggaagatgctggttccctctc

SEQ ID NO: 6 - DNA, 23 bp, artificial
  oligonucleotide for amplifying IL-1beta
cagttcagtgatcgtacaggtgc

SEQ ID NO: 7 - DNA, 29 bp, artificial
  oligonucleotide for amplifying FLT-1
tcactatggaagatctgatttcttacagt

SEQ ID NO: 8 - DNA, 25 bp, artificial
  oligonucleotide for amplifying FLT-1
ggtataaatacacatgtgcttctag

SEQ ID NO: 9 - DNA, 20 bp, artificial
  oligonucleotide for amplifying TNFalpha
tcagatcatcttctcgaacc

SEQ ID NO: 10 - DNA, 20 bp, artificial
  oligonucleotide for amplifying TNFalpha
cagatagatgggctcatacc

SEQ ID NO: 11 - DNA, 20 bp, artificial
  oligonucleotide for amplifying KDR
tatagatggtgtaacccgga

SEQ ID NO: 12 - DNA, 21 bp, artificial
  oligonucleotide for amplifying KDR
tttgtcactgagacagcttgg

SEQ ID NO: 13 - DNA, 21 bp, artificial
  oligonucleotide for amplifying RANK-ligand
aacaggcctttcaaggagctg

SEQ ID NO: 14 - DNA, 22 bp, artificial
  oligonucleotide for amplifying RANK-ligand
taaggaggggttggagacctcg

SEQ ID NO: 15 - DNA, 20 bp, artificial
  oligonucleotide for amplifying Leptin
atgcattgggaaccctgtgc

SEQ ID NO: 16 - DNA, 20 bp, artificial
  oligonucleotide for amplifying Leptin
gcacccagggctgaggtcca

SEQ ID NO: 17 - DNA, 21 bp, artificial
  oligonucleotide for amplifying CBFA-1
gtggacgaggcaagagtttca

SEQ ID NO: 18 - DNA, 21 bp, artificial
  oligonucleotide for amplifying CBFA-1
tggcaggtaggtgtggtagtg

SEQ ID NO: 19 - DNA, 28 bp, artificial
  oligonucleotide for amplifying PPARgamma2
aactgcggggaaacttgggagattctcc

SEQ ID NO: 20 - DNA, 26 bp, artificial
  oligonucleotide for amplifying PPARgamma2
aataataaggtggagatgcaggctcc

SEQ ID NO: 21 - DNA, 21 bp, artificial
  oligonucleotide for amplifying OCN
atgagagccctcacactcctc

SEQ ID NO: 22 - DNA, 19 bp, artificial
  oligonucleotide for amplifying OCN
cgtagaagcgccgataggc

SEQ ID NO: 23 - DNA, 20 bp, artificial
  oligonucleotide for amplifying MyoD
aagcgccatctcttgaggta

SEQ ID NO: 24 - DNA, 20 bp, artificial
  oligonucleotide for amplifying MyoD
gcgagaaacgtgaacctagc

SEQ ID NO: 25 - DNA, 20 bp, artificial
  oligonucleotide for amplifying SMMHC
ctgggcaacgtagtaaaacc

SEQ ID NO: 26 - DNA, 20 bp, artificial
  oligonucleotide for amplifying SMMHC
tatagctcattgcagcctcg

SEQ ID NO: 27 - DNA, 21 bp, artificial
  oligonucleotide for amplifying GFAP
ctgttgccagagatggaggtt

SEQ ID NO: 28 - DNA, 20 bp, artificial
  oligonucleotide for amplifying GFAP
tcatcgctcaggaggtcctt

SEQ ID NO: 29 - DNA, 24 bp, artificial
  oligonucleotide for amplifying nestin
ggcagcgttggaacagaggttgga

SEQ ID NO: 30 - DNA, 24 bp, artificial
  oligonucleotide for amplifying nestin
ctctaaactggagtggtcagggct

SEQ ID NO: 31 - DNA, 21 bp, artificial
  oligonucleotide for amplifying SOX9
ctctgcctgtttggactttgt

SEQ ID NO: 32 - DNA, 21 bp, artificial
  oligonucleotide for amplifying SOX9
cctttgcttgccttttacctc

SEQ ID NO: 33 - DNA, 20 bp, artificial
  oligonucleotide for amplifying collagen type X
agccagggttgccaggacca

SEQ ID NO: 34 - DNA, 20 bp, artificial
  oligonucleotide for amplifying collagen type X
ttttcccactccaggagggc

SEQ ID NO: 35 - DNA, 20 bp, artificial
  oligonucleotide for amplifying aggrecan
cactgttaccgccacttccc

SEQ ID NO: 36 - DNA, 20 bp, artificial
  oligonucleotide for amplifying aggrecan
accagcggaagtccccttcg